European Patent Specification EP 3 802 593 B1, published September 11, 2024. Title: DOSAGE AND ADMINISTRATION OF ANTI-C5 ANTIBODIES FOR TREATMENT OF PAROXYSMAL NOCTURNAL HEMOGLOBINURIA (PNH) IN PEDIATRIC PATIENTS. Applicant: ALEXION PHARMACEUTICALS, INC. The sequence listing filed with the application follows.

SEQUENCE LISTING (46 sequences)

SEQ ID NO: 1 - protein, 10 aa, Artificial Sequence
  source: /note="Description of Artificial Sequence: Synthetic peptide"
GYIFSNYWIQ

SEQ ID NO: 2 - protein, 17 aa, Artificial Sequence
  source: /note="Description of Artificial Sequence: Synthetic peptide"
EILPGSGSTEYTENFKD

SEQ ID NO: 3 - protein, 13 aa, Artificial Sequence
  source: /note="Description of Artificial Sequence: Synthetic peptide"
YFFGSSPNWYFDV

SEQ ID NO: 4 - protein, 11 aa, Artificial Sequence
  source: /note="Description of Artificial Sequence: Synthetic peptide"
GASENIYGALN

SEQ ID NO: 5 - protein, 7 aa, Artificial Sequence
  source: /note="Description of Artificial Sequence: Synthetic peptide"
GATNLAD

SEQ ID NO: 6 - protein, 9 aa, Artificial Sequence
  source: /note="Description of Artificial Sequence: Synthetic peptide"
QNVLNTPLT

SEQ ID NO: 7 - protein, 122 aa, Artificial Sequence [sequence omitted]

SEQ ID NO: 8 - protein, 107 aa, Artificial Sequence [sequence omitted]

SEQ ID NO: 9 - protein, 326 aa, Artificial Sequence
  source: /note="Description of Artificial Sequence: Synthetic polypeptide"
ASTKGPSVFPLAPCSRSTSESTAALGCLVKDYFPEPVTVSWNSGALTSGVHTFPAVLQSSGLYSLSSVVTVPSSNFGTQTYTCNVDHKPSNTKVDKTVERKCCVECPPCPAPPVAGPSVFLFPPKPKDTLMISRTPEVTCVVVDVSQEDPEVQFNWYVDGVEVHNAKTKPREEQFNSTYRVVSVLTVLHQDWLNGKEYKCKVSNKGLPSSIEKTISKAKGQPREPQVYTLPPSQEEMTKNQVSLTCLVKGFYPSDIAVEWESNGQPENNYKTTPPVLDSDGSFFLYSRLTVDKSRWQEGNVFSCSVMHEALHNHYTQKSLSLSLGK

SEQ ID NO: 10 - protein, 447 aa, Artificial Sequence
  source: /note="Description of Artificial Sequence: Synthetic polypeptide"
QVQLVQSGAEVKKPGASVKVSCKASGYIFSNYWIQWVRQAPGQGLEWMGEILPGSGSTEYTENFKDRVTMTRDTSTSTVYMELSSLRSEDTAVYYCARYFFGSSPNWYFDVWGQGTLVTVSSASTKGPSVFPLAPCSRSTSESTAALGCLVKDYFPEPVTVSWNSGALTSGVHTFPAVLQSSGLYSLSSVVTVPSSNFGTQTYTCNVDHKPSNTKVDKTVERKCCVECPPCPAPPVAGPSVFLFPPKPKDTLMISRTPEVTCVVVDVSQEDPEVQFNWYVDGVEVHNAKTKPREEQFNSTYRVVSVLTVLHQDWLNGKEYKCKVSNKGLPSSIEKTISKAKGQPREPQVYTLPPSQEEMTNQVSLTCLVKGFYPSDIAVEWESNGQPENNYKTTPPVLDSDGSFFLYSRLTVDKSRWQEGNVFSCSVMHEALHNHYTQKSLSLSLGK

SEQ ID NO: 11 - protein, 214 aa, Artificial Sequence [sequence omitted]

SEQ ID NO: 12 - protein, 122 aa, Artificial Sequence [sequence omitted]

SEQ ID NO: 13 - protein, 326 aa, Artificial Sequence
  source: /note="Description of Artificial Sequence: Synthetic polypeptide"
ASTKGPSVFPLAPCSRSTSESTAALGCLVKDYFPEPVTVSWNSGALTSGVHTFPAVLQSSGLYSLSSVVTVPSSNFGTQTYTCNVDHKPSNTKVDKTVERKCCVECPPCPAPPVAGPSVFLFPPKPKDTLMISRTPEVTCVVVDVSQEDPEVQFNWYVDGVEVHNAKTKPREEQFNSTYRVVSVLTVLHQDWLNGKEYKCKVSNKGLPSSIEKTISKAKGQPREPQVYTLPPSQEEMTKNQVSLTCLVKGFYPSDIAVEWESNGQPENNYKTTPPVLDSDGSFFLYSRLTVDKSRWQEGNVFSCSVLHEALHSHYTQKSLSLSLGK

SEQ ID NO: 14 - protein, 448 aa, Artificial Sequence
  source: /note="Description of Artificial Sequence: Synthetic polypeptide"
QVQLVQSGAEVKKPGASVKVSCKASGHIFSNYWIQWVRQAPGQGLEWMGEILPGSGHTEYTENFKDRVTMTRDTSTSTVYMELSSLRSEDTAVYYCARYFFGSSPNWYFDVWGQGTLVTVSSASTKGPSVFPLAPCSRSTSESTAALGCLVKDYFPEPVTVSWNSGALTSGVHTFPAVLQSSGLYSLSSVVTVPSSNFGTQTYTCNVDHKPSNTKVDKTVERKCCVECPPCPAPPVAGPSVFLFPPKPKDTLMISRTPEVTCVVVDVSQEDPEVQFNWYVDGVEVHNAKTKPREEQFNSTYRVVSVLTVLHQDWLNGKEYKCKVSNKGLPSSIEKTISKAKGQPREPQVYTLPPSQEEMTKNQVSLTCLVKGFYPSDIAVEWESNGQPENNYKTTPPVLDSDGSFFLYSRLTVDKSRWQEGNVFSCSVLHEALHSHYTQKSLSLSLGK

SEQ ID NO: 15 - protein, 326 aa, Artificial Sequence
  source: /note="Description of Artificial Sequence: Synthetic polypeptide"
ASTKGPSVFPLAPCSRSTSESTAALGCLVKDYFPEPVTVSWNSGALTSGVHTFPAVLQSSGLYSLSSVVTVTSSNFGTQTYTCNVDHKPSNTKVDKTVERKCCVECPPCPAPPVAGPSVFLFPPKPKDTLYITREPEVTCVVVDVSHEDPEVQFNWYVDGMEVHNAKTKPREEQFNSTFRVVSVLTVVHQDWLNGKEYKCKVSNKGLPAPIEKTISKTKGQPREPQVYTLPPSREEMTKNQVSLTCLVKGFYPSDIAVEWESNGQPENNYKTTPPMLDSDGSFFLYSKLTVDKSRWQQGNVFSCSVMHEALHNHYTQKSLSLSPGK

SEQ ID NO: 16 - protein, 448 aa, Artificial Sequence
  source: /note="Description of Artificial Sequence: Synthetic polypeptide"
QVQLVQSGAEVKKPGASVKVSCKASGYIFSNYWIQWVRQAPGQGLEWMGEILPGSGSTEYTENFKDRVTMTRDTSTSTVYMELSSLRSEDTAVYYCARYFFGSSPNWYFDVWGQGTLVTVSSASTKGPSVFPLAPCSRSTSESTAALGCLVKDYFPEPVTVSWNSGALTSGVHTFPAVLQSSGLYSLSSVVTVTSSNFGTQTYTCNVDHKPSNTKVDKTVERKCCVECPPCPAPPVAGPSVFLFPPKPKDTLYITREPEVTCVVVDVSHEDPEVQFNWYVDGMEVHNAKTKPREEQFNSTFRVVSVLTVVHQDWLNGKEYKCKVSNKGLPAPIEKTISKTKGQPREPQVYTLPPSREEMTKNQVSLTCLVKGFYPSDIAVEWESNGQPENNYKTTPPMLDSDGSFFLYSKLTVDKSRWQQGNVFSCSVMHEALHNHYTQKSLSLSPGK

SEQ ID NO: 17 - protein, 11 aa, Artificial Sequence
  source: /note="Description of Artificial Sequence: Synthetic peptide"
GASENIYHALN

SEQ ID NO: 18 - protein, 17 aa, Artificial Sequence
  source: /note="Description of Artificial Sequence: Synthetic peptide"
EILPGSGHTEYTENFKD

SEQ ID NO: 19 - protein, 10 aa, Artificial Sequence
  source: /note="Description of Artificial Sequence: Synthetic peptide"
GHIFSNYWIQ

SEQ ID NO: 20 - protein, 448 aa, Artificial Sequence
  source: /note="Description of Artificial Sequence: Synthetic polypeptide"
QVQLVQSGAEVKKPGASVKVSCKASGHIFSNYWIQWVRQAPGQGLEWMGEILPGSGHTEYTENFKDRVTMTRDTSTSTVYMELSSLRSEDTAVYYCARYFFGSSPNWYFDVWGQGTLVTVSSASTKGPSVFPLAPCSRSTSESTAALGCLVKDYFPEPVTVSWNSGALTSGVHTFPAVLQSSGLYSLSSVVTVPSSNFGTQTYTCNVDHKPSNTKVDKTVERKCCVECPPCPAPPVAGPSVFLFPPKPKDTLMISRTPEVTCVVVDVSQEDPEVQFNWYVDGVEVHNAKTKPREEQFNSTYRVVSVLTVLHQDWLNGKEYKCKVSNKGLPSSIEKTISKAKGQPREPQVYTLPPSQEEMTKNQVSLTCLVKGFYPSDIAVEWESNGQPENNYKTTPPVLDSDGSFFLYSRLTVDKSRWQEGNVFSCSVMHEALHNHYTQKSLSLSLGK

SEQ ID NO: 21 - protein, 5 aa, Artificial Sequence
  source: /note="Description of Artificial Sequence: Synthetic peptide"
SYAIS

SEQ ID NO: 22 - protein, 17 aa, Artificial Sequence
  source: /note="Description of Artificial Sequence: Synthetic peptide"
GIGPFFGTANYAQKFQG

SEQ ID NO: 23 - protein, 7 aa, Artificial Sequence
  source: /note="Description of Artificial Sequence: Synthetic peptide"
DTPYFDY

SEQ ID NO: 24 - protein, 11 aa, Artificial Sequence
  source: /note="Description of Artificial Sequence: Synthetic peptide"
SGDSIPNYYVY

SEQ ID NO: 25 - protein, 7 aa, Artificial Sequence
  source: /note="Description of Artificial Sequence: Synthetic peptide"
DDSNRPS

SEQ ID NO: 26 - protein, 11 aa, Artificial Sequence
  source: /note="Description of Artificial Sequence: Synthetic peptide"
QSFDSSLNAEV

SEQ ID NO: 27 - protein, 116 aa, Artificial Sequence
  source: /note="Description of Artificial Sequence: Synthetic polypeptide"
QVQLVQSGAEVKKPGSSVKVSCKASGGTFSSYAISVWRQAPGQGLEWMGGIGPFFGTANYAQKFQGRVTITADESTSTAYMELSSLRSEDTAVYYCARDTPYFDYWGQGTLVTVSS

SEQ ID NO: 28 - protein, 108 aa, Artificial Sequence
  source: /note="Description of Artificial Sequence: Synthetic polypeptide"
DIELTQPPSVSVAPGQTARISCSGDSIPNYYVYWYQQKPGQAPVLVIYDDSNRPSGIPERFSGSNSGNTATLTISGTQAEDEADYYCQSFDSSLNAEVFGGGTKLTVL

SEQ ID NO: 29 - protein, 4 aa, Artificial Sequence
  source: /note="Description of Artificial Sequence: Synthetic peptide"
NYIS

SEQ ID NO: 30 - protein, 17 aa, Artificial Sequence
  source: /note="Description of Artificial Sequence: Synthetic peptide"
IIDPDDSYTEYSPSFQG

SEQ ID NO: 31 - protein, 8 aa, Artificial Sequence
  source: /note="Description of Artificial Sequence: Synthetic peptide"
YEYGGFDI

SEQ ID NO: 32 - protein, 11 aa, Artificial Sequence
  source: /note="Description of Artificial Sequence: Synthetic peptide"
SGDNIGNSYVH

SEQ ID NO: 33 - protein, 7 aa, Artificial Sequence
  source: /note="Description of Artificial Sequence: Synthetic peptide"
KDNDRPS

SEQ ID NO: 34 - protein, 9 aa, Artificial Sequence
  source: /note="Description of Artificial Sequence: Synthetic peptide"
GTYDIESYV

SEQ ID NO: 35 - protein, 116 aa, Artificial Sequence
  source: /note="Description of Artificial Sequence: Synthetic polypeptide"
EVQLVQSGAEVKKPGESLKISCKGSGYSFTNYISWVRQMPGKGLEWMGIIDPDDSYTEYSPSFQGQVTISADKSISTAYLQWSSLKASDTAMYYCARYEYGGFDIWGQGTLVTVSS

SEQ ID NO: 36 - protein, 106 aa, Artificial Sequence
  source: /note="Description of Artificial Sequence: Synthetic polypeptide"
SYELTQPPSVSVAPGQTARISCSGDNIGNSYVHWYQQKPGQAPVLVIYKDNDRPSGIPERFSGSNSGNTATLTISGTQAEDEADYYCGTYDIESYVFGGGTKLTVL

SEQ ID NO: 37 - protein, 6 aa, Artificial Sequence
  source: /note="Description of Artificial Sequence: Synthetic peptide"
SSYYVA

SEQ ID NO: 38 - protein, 17 aa, Artificial Sequence
  source: /note="Description of Artificial Sequence: Synthetic peptide"
AIYTGSGATYKASWAKG

SEQ ID NO: 39 - protein, 13 aa, Artificial Sequence
  source: /note="Description of Artificial Sequence: Synthetic peptide"
DGGYDYPTHAMHY

SEQ ID NO: 40 - protein, 11 aa, Artificial Sequence
  source: /note="Description of Artificial Sequence: Synthetic peptide"
QASQNIGSSLA

SEQ ID NO: 41 - protein, 7 aa, Artificial Sequence
  source: /note="Description of Artificial Sequence: Synthetic peptide"
GASKTHS

SEQ ID NO: 42 - protein, 12 aa, Artificial Sequence
  source: /note="Description of Artificial Sequence: Synthetic peptide"
QSTKVGSSYGNH

SEQ ID NO: 43 - protein, 123 aa, Artificial Sequence
  source: /note="Description of Artificial Sequence: Synthetic polypeptide"
QVQLVESGGGLVQPGGSLRLSCAASGFTSHSSYYVAWVRQAPGKGLEWVGAIYTGSGATYKASWAKGRFTISKDTSKNQVVLTMTNMDPVDTATYYCASDGGYDYPTHAMHYWGQGTLVTVSS

SEQ ID NO: 44 - protein, 110 aa, Artificial Sequence
  source: /note="Description of Artificial Sequence: Synthetic polypeptide"
DVVMTQSPSSLSASVGDRVTITCQASQNIGSSLAWYQQKPGQAPRLLIYGASKTHSGVPSRFSGSGSGTDFTLTISSLQPEDVATYYCQSTKVGSSYGNHFGGGTKVEIK

SEQ ID NO: 45 - protein, 451 aa, Artificial Sequence
  source: /note="Description of Artificial Sequence: Synthetic polypeptide"
QVQLVESGGGLVQPGRSLRLSCAASGFTVHSSYYMAWVRQAPGKGLEWVGAIFTGSGAEYKAEWAKGRVTISKDTSKNQVVLTMTNMDPVDTATYYCASDAGYDYPTHAMHYWGQGTLVTVSSASTKGPSVFPLAPSSKSTSGGTAALGCLVKDYFPEPVTVSWNSGALTSGVHTFPAVLQSSGLYSLSSVVTVPSSSLGTQTYICNVNHKPSNTKVDKKVEPKSCDKTHTCPPCPAPELRRGPKVFLFPPKPKDTLMISRTPEVTCVVVDVSHEDPEVKFNWYVDGVEVHNAKTKPREEQYNSTYRVVSVLTVLHQDWLNGKEYKCKVSNKGLPSSIEKTISKAKGQPREPQVYTLPPSREEMTKNQVSLTCLVKGFYPSDIAVEWESNGQPENNYKTTPPVLDSDGSFFLYSKLTVDKSRWQQGNVFSCSVLHEALHAHYTRKELSLSP

SEQ ID NO: 46 - protein, 217 aa, Artificial Sequence
  source: /note="Description of Artificial Sequence: Synthetic polypeptide"
DIQMTQSPSSLSASVGDRVTITCRASQGISSSLAWYQQKPGKAPKLLIYGASETESGVPSRFSGSGSGTDFTLTISSLQPEDFATYYCQNTKVGSSYGNTFGGGTKVEIKRTVAAPSVFIFPPSDEQLKSGTASVVCLLNNFYPREAKVQWKVDNALQSGNSQESVTEQDSKDSTYSLSSTLTLSKADYEKHKVYACEVTHQGLSSPVTKSFNRGEC